European Patent Application EP 4 509 610 A1, published February 19, 2025. Title: 一种制备酮酸的方法及该方法在制备氨基酸或氨基酸衍生物中的应用. Applicant: 元素驱动（杭州）生物科技有限公司. The sequence listing filed with the application follows.

SEQUENCE LISTING (9 sequences)

SEQ ID NO: 1 - DNA, 1041 bp, Pseudomonas putida
  source 1..1041: mol_type = genomic DNA
atgacagacaagagccaacaattcgccagcgacaactattccggtatctgccccgaagcctgggtggcgatggagaaagccaaccgcggccacgaccgcgcctacggcgacgaccagtggaccgagcgtgcatcggagtacttccgcaatctgttcgaaaccgactgcgaggtgttctttgccttcaacggcaccgcggccaactccctggccctggcatccctgtgccagagctatcacagcgtgatctgctccgagaccgcccacgtcgaaaccgacgaatgcggtgcaccggagtttttctccaacggctccaagctgctgacggcggccagcgtcaacggcaagctgacgccacagtcgatccgcgaagtggcgctcaaacgccaggatatccactaccccaagccgcgcgtggtgaccattacccaggccaccgaagtgggcacggtgtaccgccccgacgagctgaaggcgatcagcgccacctgcaaggagctgggcctgaacctgcacatggacggcgcacgctttaccaatgcctgtgcgttcctgggctgcagcccggccgaactgacctggaaggccggtgtggatgtgctgtgctttggcggcaccaagaacggcatggcggtgggcgaagcgattctgttcttcaaccgccagctggccgaagacttcgattatcgctgcaagcaggccgggcaactggcgtcgaagatgcgcttcttgtcggcgccctgggtcgggctgctggaagatggcgcatggttacgccatggcaaccacgccaatcattgcgcgcaactgctggcatcgctggtcagtgacctgccgggggtagagctgatgttcccggtggaggccaacggggtgttcctgcagatgccagagcacgccatcgaggcgctgcggggcaagggctggcgcttctatacctttatcggcagcggtggcgcgcgcttcatgtgctcgtgggataccgaagaagcgcgggtgcgtgagctggcggcggatatccgcacgatcattggtggctga

SEQ ID NO: 2 - DNA, 1002 bp, Escherichia coli
  source 1..1002: mol_type = genomic DNA
atgattgatttacgcagtgataccgttacccgaccaagccgcgccatgctcgaagcgatgatggccgccccggttggggacgacgtttacggagacgaccctaccgttaatgctctgcaggactacgcagcagagctttccggtaaagaagccgccatttttctgcctaccggcactcaggccaacctggtcgctctgctcagtcactgcgaacgcggcgaagagtatattgtcggtcaggccgcgcataactatctgtttgaagccggtggcgcggcggtgctgggcagtattcaaccgcaacccatagacgcggctgccgacggcacgctaccgctggataaagtggcgatgaaaatcaaacccgacgatatccatttcgcccgcaccaaattactcagtctggaaaacacccacaacggcaaagtgttgccgcgggaatacctgaaagaagcatgggaatttacccgcgagcgcaatctggcgctgcatgttgacggtgcgcgcatctttaatgccgtggtggcttacggctgcgaactgaaagagatcacgcaatattgtgattcgttcaccatttgcctgtcgaaaggtcttgggacgccagtcggttcattactcgtcggtaatcgtgattacattaaacgtgccattcgctggcggaaaatgacaggtggcgggatgcgccagtccggcattctggctgccgccgggatatatgccctgaaaaataacgttgcgcgcttgcaggaagaccacgacaacgctgcctggatggcggagcagctgcgtgaagcaggcgcggatgtgatgcgtcaggacaccaatatgctgtttgttcgcgtcggggaagaaaatgctgccgcgttaggcgaatacatgaaagcgagaaacgtgctgattaacgcctcgccgattgtccgcctggtgacgcatcttgacgtctcgcgcgaacaactggcggaagtcgccgcccactggcgtgcattcctggcgcgttaa

SEQ ID NO: 3 - DNA, 1545 bp, Escherichia coli
  source 1..1545: mol_type = genomic DNA
atggctgactcgcaacccctgtccggtgctccggaaggtgccgaatatttaagagcagtgctgcgcgcgccggtttacgaggcggcgcaggttacgccgctacaaaaaatggaaaaactgtcgtcgcgtcttgataacgtcattctggtgaagcgcgaagatcgccagccagtgcacagctttaagctgcgcggcgcatacgccatgatggcgggcctgacggaagaacagaaagcgcacggcgtgatcactgcttctgcgggtaaccacgcgcagggcgtcgcgttttcttctgcgcggttaggcgtgaaggccctgatcgttatgccaaccgccaccgccgacatcaaagtcgacgcggtgcgcggcttcggcggcgaagtgctgctccacggcgcgaactttgatgaagcgaaagccaaagcgatcgaactgtcacagcagcaggggttcacctgggtgccgccgttcgaccatccgatggtgattgccgggcaaggcacgctggcgctggaactgctccagcaggacgcccatctcgaccgcgtatttgtgccagtcggcggcggcggtctggctgctggcgtggcggtgctgatcaaacaactgatgccgcaaatcaaagtgatcgccgtagaagcggaagactccgcctgcctgaaagcagcgctggatgcgggtcatccggttgatctgccgcgcgtagggctatttgctgaaggcgtagcggtaaaacgcatcggtgacgaaaccttccgtttatgccaggagtatctcgacgacatcatcaccgtcgatagcgatgcgatctgtgcggcgatgaaggatttattcgaagatgtgcgcgcggtggcggaaccctctggcgcgctggcgctggcgggaatgaaaaaatatatcgccctgcacaacattcgcggcgaacggctggcgcatattctttccggtgccaacgtgaacttccacggcctgcgctacgtctcagaacgctgcgaactgggcgaacagcgtgaagcgttgttggcggtgaccattccggaagaaaaaggcagcttcctcaaattctgccaactgcttggcgggcgttcggtcaccgagttcaactaccgttttgccgatgccaaaaacgcctgcatctttgtcggtgtgcgcctgagccgcggcctcgaagagcgcaaagaaattttgcagatgctcaacgacggcggctacagcgtggttgatctctccgacgacgaaatggcgaagctacacgtgcgctatatggtcggcggacgtccatcgcatccgttgcaggaacgcctctacagcttcgaattcccggaatcaccgggcgcgctgctgcgcttcctcaacacgctgggtacgtactggaacatttctttgttccactatcgcagccatggcaccgactacgggcgcgtactggcggcgttcgaacttggcgaccatgaaccggatttcgaaacccggctgaatgagctgggctacgattgccacgacgaaaccaataacccggcgttcaggttctttttggcgggttag

SEQ ID NO: 4 - DNA, 1032 bp, Burkholderia thailandensis
  source 1..1032: mol_type = genomic DNA
atgtcgacctcaccccaccgccccgctcatctgacgatcaacggcgagccgattccgacgctcgacgaaatcgccgcgcagcacttcgcgctcacgccgtgggtcacgcgtacgccggtgttcgagcgcgccgatctgccatcgctcgacaacacgcacgtgaacttcaagttcgagctgctgcaggcgagcggcagcttcaaggcgcgcggcgcgttcacgaacctgctcgcgctcggcgaggacagaaagcgcgcgggcgtcacctgcgtgtcggcgggcaatcatgcggcggccgtcgcttatgcggcgatgcggctcggcacgagcgcgaaggtcgtgatgttcgacaccgcgagcccggcgcgcgtcgagctctgccaccagtaccgcgcggaggtcgtgatggcgtcgagccccgccgacgcgttcgagatcgtccggcgaatcgaggccgaggaaggccgcttcttcgtgcatccgttcaacggctatcacacgattctcggcaccgcgacgctcggctacgaatgggcgacgcagacgcccgacctcgatgcggtgatcgtgccgatcggcggcggcggcctcgccgcgggcacctcgaccgcgctgcggcttgcgaatccgcgcgtgcacgtgtacggcgtcgagccggaaggtgcggatgtgatgagccgcagcttcgccgcgaatcgcccggtccgcatgggcgcgatgcatacgatcgccgattcgctgatggcgccgcacaccgaggagtacagctacgagctgtgccgccgccatgtcgaccggatcgtcaccgtctcggacgacgcgctgcgagcggcgatgctctatttgttcacgcatctgaaagtggcggtcgagcccgcgtgcgcggccgcgacggccgccctcctcgggccgttgcgcgagtcgctgcaaggcaagcgtgttggcgtgctgctgtcgggcaccaacatcgattcgacggcgctcgccacgcatctcgagcatgctcggctgcatcgcatgtcgtggccgtga

SEQ ID NO: 5 - DNA, 387 bp, Escherichia coli
  source 1..387: mol_type = genomic DNA
atgagcaaaactatcgcgacggaaaatgcaccggcagctatcggtccttacgtacagggcgttgatctgggcaatatgatcatcacctccggtcagatcccggtaaatccgaaaacgggcgaagtaccggcagacgtcgctgcacaggcacgtcagtcgctggataacgtaaaagcgatcgtcgaagccgctggcctgaaagtgggcgacatcgttaaaactaccgtgtttgtaaaagatctgaacgacttcgcaaccgtaaacgccacttacgaagccttcttcaccgaacacaacgccaccttcccggcacgttcttgcgttgaagttgcccgtctgccgaaagacgtgaagattgagatcgaagcgatcgctgttcgtcgctaa

SEQ ID NO: 6 - DNA, 1479 bp, Pseudomonas putida
  source 1..1479: mol_type = genomic DNA
atggcggtatttgccagtgactcttttggccagctgaaagtggagaaaattatgactgcccagtggaaccactacattaacggggaatacgtatcacccgaatctgaagagtatatccacgagttcatcccaaccacggctttgccgggtgactcaatcgcaaggggctcggcagctgacgttgataaggctgttcgtgccgcggcagcggctcagcctgcctggaatgcacgcaagccaattgagcggggtcgtatccttctcgccatagctcgtttggttcgcgccaacgcagcggctttctgcgccaaagaagcggaagaaactggcaagcctctgaagatggccgcctttgagatcgaggcatgtgctcagtactttgagtattacggcggtttggcgacagccatccagggcgaaaccatcaacctcggccccagctaccacgcctataccacccgagagccatttggagtggtgggggtcatcctgccgtggaattcgccactgaaccaagctgggcgagccattgccccggcattggttagcgggaacaccgtggtggtcaaaccttcagagttcacctcggtgacgatgctccagttcgcggaactggttgtgaaagaggcagggttgccaccaggcgtattgaacgtggttaccggcaccggtaaggaaaccggtgagcctctggttaaacaccctctgatccgaaaggttgctttcaccggttctgtccgtgccggacgggagatcggcaagctcgccgcagatcgcatcattccgctgtcgctcgaattgggcggcaaatccccgaacattgtcttcgaagacgcagatctggatcgagctgtcgcgggtagcgtctttgccttcaccgtcaacactggtcaagtctgtctcgccgggacccgttgcctggtgcatgagtcgatttttgaaaaattctccaagaagcttgccggtgctgtagaggcgcttcagttcagcgacggcgaaagcttcggtctcggccccctaacgaccaaggctcagtttgagcaggttcatcgttacaacgagctggccatccaggagggggctcattgcttggtcggtggggaagctccaagtgacaaaaccggctggtacgtacgacccaccgtctacaccaacgtcaacaactcgatgcggattgctcgggaagaaattttcggacccgttctggtactgattccgttcaaggacgaaaacgaggcggtggccatcgcgaatgactcggactacgggctcgcggctggcgtatggaccaccgatctggctcgcgcgcaccgcgtatccgctcaaatcgaagcgggccaggtgtacgtcaacgaatatccatcaggtggcgttgagactccattcggcggtttcaagcaaagcggccatgggcgcgagaagggcattgaagcactccaccattacacccaaacaaagacgaccatcatccgcatttaa

SEQ ID NO: 7 - DNA, 1287 bp, Chlamydomonas reinhardtii
  source 1..1287: mol_type = genomic DNA
atgcgcgcactggttagcaaagcacgcctggcacatagcgtgggtggtcgtgcgagccaggcgacccgttgcgcagcaaccattagcgcaagccgtgcaccggcccatctgggtgatgccctgcatgatgttgataccccggcactgattctggatctggatgcatttgatcgtaactgtgaaaaactgaaaggtgttatggcaggttttcctggtgttgcagttcgtccgcatgcaaaagcacataaatgtgcagaagttgcccgccgtcagctgcagctgctgggtgctaaaggtgtttgctgtcagaaagttattgaagcggaagcaatggcagaaggtggtgtttccgatctgctgctgagcaatgaagtgattgcacctcgtaaaatcgatcgtctggttggtctggcagcggccggtgcacgcgttggtgtgtgttatgaacgtgaagataatctgcgtcagctgaatgccgcagcagcagcacgtggtacacatctggatgttctggttgaactgaatgttggtcaggatcgttgtggtgttaatagcgccgatgaagttgttcagctggcccgtgcagccgccggtctggataatgttcgttttgcaggtattcaggcatatcatggtggtctgcagcatgttcgtgatccgcgtgatcgcgcacagcgtgttggtcaggttgttggtcgtgcacgtgcagcagttgatgcgctgaaagcagcaggtctgccatgtgataccgttacaggtggtggtacaggtacatatcgtgtggaagcagcaagtggtgtttttacggaagttcagccgggtagttttgcattttctgatgccgattatgcgcgtaatctgcaggaagatggtggtgtgggtgaatgggaacagagcctgtgggttctgacccaggtgatgagcgtgaccccggcacgtggtctggcagttgttgatgcaggtacaaaagcagtgtctctggatagtggtccgccgcgtctgccgccggcatttgaagctgcatacggtacaatgatggaatatggctctggtggtgatgaacatggtaaactgatgtggccgcagggtgcgtatcagctgccgatgtcactgcctgaagttggtagcctgctgctgctgcagccgggtcattgtgatccgacagttaatctgtatgattggctggtggccgcgcgtcgtcagcagggtggtcagcagcagggtggcgttgatggttggcgtgttgaagcagtttggccgattcgtggtcgtggtcctggccagtga

SEQ ID NO: 8 - DNA, 1353 bp, Lactobacillus buchneri
  source 1..1353: mol_type = genomic DNA
atgggcaaactggacaaagcgagcaaactgatcgacgaagaaaataaatactacgcacgtagcgcgcgtatcaactactacaacctggtgattgaccacgcccacggcgcaaccctggtggatgtggatggaaataaatatatcgatctgctggcaagcgcaagcgcaattaatgttggtcatacccatgaaaaagttgtgaaagcaattgcagatcaagcacaaaaactgattcattataccccggcatacttccaccacgttccgggtatggaactgagcgaaaaactggcaaaaattgcaccgggtaatagccctaaaatggtgagttttggaaatagcggaagcgatgcaaatgatgcaattatcaaatttgcacgtgcatatacgggacgtcagtatattgttagttacatgggtagctatcacggaagcacctacggtagccagacactgtcaggttcaagcctgaatatgacccgcaaaatcggtccgatgctgccgagcgttgttcatgttccgtatccggattcatatcgcacctacccgggagaaactgagcacgatgttagcctgcgttattttaatgagtttaaaaagccgttcgagagctttctgcctgcagatgagaccgcatgtgttctgattgaaccgattcagggcgatggaggtattattaaagcaccggaagaatatatgcagctggtgtataaattttgtcatgaacatggtatcctgtttgcaattgatgaagttaatcaaggcctgggtcgtacaggaaaaatgtgggcaatccagcagtttaaagatattgaaccggatctgatgagcgttggtaaaagcctggcgtctggtatgccgctgagcgcagttatcggtaaaaaggaagttatgcagagcctggacgcacctgcacacctgtttaccaccgcaggtaatccggtttgtagtgcagcaagcctggcaactctggacgttattgaatatgaggggctggtggagaaaagcgcaaccgacggtgcatatgccaaacaacgttttctggaaatgcaacagcgccatccgatgatcggagatgttcgtatgtgggggctgaatgggggtattgaactggttaaagacccgaaaaccaaagaacctgatagtgacgcagcaaccaaagtgatttactacgcctttgcacacggggttgtaattattacgctggcaggcaacattctgcgctttcaaccgccgctggttatcccgcgtgaacaactggatcaggcactgcaggtgctggatgacgcctttaccgcagtcgaaaatggggaagttaccattccgaaagacaccggtaaaattggctggtaa

SEQ ID NO: 9 - DNA, 1143 bp, Bacillus badius
  source 1..1143: mol_type = genomic DNA
atgagcctggtggaaaaaaccagcattattaaagattttaccctgtttgaaaaaatgagcgaacatgaacaggttgttttttgtaatgatccggcaaccggtctgcgtgcaattattgcaattcatgataccaccctgggtccggcactgggtggttgtcgtatgcagccgtataatagcgttgaagaagcactggaagatgcactgcgtctgagcaaaggtatgacctataaatgtgcagcaagcgatgttgattttggtggtggtaaagcagttattattggtgatccgcagaaagataaaagcccggaactgtttcgtgcatttggtcagtttgttgatagcctgggtggtcgtttttataccggtaccgatatgggtaccaatatggaagattttattcatgcaatgaaagaaaccaattgtattgttggtgttccggaagcatatggtggtggtggtgatagcagcattccgaccgcaatgggtgttctgtatggtattaaagcaaccaataaaatgctgtttggtaaagatgatctgggtggtgttacctatgcaattcagggtctgggtaaagttggttataaagttgcagaaggtctgctggaagaaggtgcacatctgtttgttaccgatattaatgaacagaccctggaagcaattcaggaaaaagcaaaaaccaccagcggtagcgttaccgttgttgcaagcgatgaaatttatagccaggaagcagatgtttttgttccgtgtgcatttggtggtgttgttaatgatgaaaccatgaaacagtttaaagttaaagcaattgcaggtagcgcaaataatcagctgctgaccgaagatcatggtcgtcatctggcagataaaggtattctgtatgcaccggattatattgttaatagcggtggtctgattcaggttgcagatgaactgtatgaagttaataaagaacgtgttctggcaaaaaccaaacatatttatgatgcaattctggaagtttatcagcaggcagaactggatcagattaccaccatggaagcagcaaatcgtatgtgtgaacagcgtatggcagcacgtggtcgtcgtaatagcttttttaccagcagcgttaaaccgaaatgggatattcgtaattaa